European Patent Specification EP 3 848 462 B1, published May 27, 2026. Title: Baicalein- and Wild Baicalein-Synthesizing Microorganism, Preparation Method For Same, and Applications Thereof. Applicant: Shanghai Institute of life sciences, Chinese Academy of Sciences. The sequence listing filed with the application follows.

SEQUENCE LISTING (29 sequences)

SEQ ID NO: 1 - protein, 517 aa, Scutellaria baicalensis
MELSSVIYGAIALLSLFYCYLHFSKPKKSSLNAPPEAGGARFITGHLHLMDGRSASDKLPHINLGLLADQHGPIFTIRLGVHRAVVVSSWELAKEIFTTHDTAVMARPRLIADDYLSYDGASLGFSPYGPYWREIRKLVTTELLSARRIELQRATRVREITQFTGELYKLWEEKKDGSGRVLVDMKQWLGNLSLNLVSRMVVGKRFYGGDDSETTKRWRGVMREFFQLIGQFIPGDGLPFLRWLDLGGFEKRTRDTAYELDKIIAMWLAEYRKREYSGDDKEQCFMALMLSLVQANPTLQLHYDADTIIKATCQVLISAASDTTTVILIWVISLLLNNADVLKKVQEELDEQVGRERRVEESDISNLPYLQAVVKETMRLYPPAPFAGVRAFSEDCTVGGYHIQKGTFLIVNLWKLHRDPRVWSDDALEFKPQRFFDKKVEVKGQDFELMPFGGGRRMCPGSNLGMHMVHFVLANILQAFDITTGSTVDMTESVGLTNMKATPLDAILTPRLSPTLY

SEQ ID NO: 2 - protein, 495 aa, Artificial Sequence
  VARIANT (1)..(495): F6H mutant
MAMPKKSSLNAPPEAGGARFITGHLHLMDGRSASDKLPHINLGLLADQHGPIFTIRLGVHRAVVVSSWELAKEIFTTHDTAVMARPRLIADDYLSYDGASLGFSPYGPYWREIRKLVTTELLSARRIELQRATRVREITQFTGELYKLWEEKKDGSGRVLVDMKQWLGNLSLNLVSRMVVGKRFYGGDDSETTKRWRGVMREFFQLIGQFIPGDGLPFLRWLDLGGFEKRTRDTAYELDKIIAMWLAEYRKREYSGDDKEQCFMALMLSLVQANPTLQLHYDADTIIKATCQVLISAASDTTTVILIWVISLLLNNADVLKKVQEELDEQVGRERRVEESDISNLPYLQAVVKETMRLYPPAPFAGVRAFSEDCTVGGYHIQKGTFLIVNLWKLHRDPRVWSDDALEFKPQRFFDKKVEVKGQDFELMPFGGGRRMCPGSNLGMHMVHFVLANILQAFDITTGSTVDMTESVGLTNMKATPLDAILTPRLSPTLY

SEQ ID NO: 3 - protein, 501 aa, Artificial Sequence
  VARIANT (1)..(501): F6H mutant 8RPtrF6H
MALLLAVFMPKKSSLNAPPEAGGARFITGHLHLMDGRSASDKLPHINLGLLADQHGPIFTIRLGVHRAVVVSSWELAKEIFTTHDTAVMARPRLIADDYLSYDGASLGFSPYGPYWREIRKLVTTELLSARRIELQRATRVREITQFTGELYKLWEEKKDGSGRVLVDMKQWLGNLSLNLVSRMVVGKRFYGGDDSETTKRWRGVMREFFQLIGQFIPGDGLPFLRWLDLGGFEKRTRDTAYELDKIIAMWLAEYRKREYSGDDKEQCFMALMLSLVQANPTLQLHYDADTIIKATCQVLISAASDTTTVILIWVISLLLNNADVLKKVQEELDEQVGRERRVEESDISNLPYLQAVVKETMRLYPPAPFAGVRAFSEDCTVGGYHIQKGTFLIVNLWKLHRDPRVWSDDALEFKPQRFFDKKVEVKGQDFELMPFGGGRRMCPGSNLGMHMVHFVLANILQAFDITTGSTVDMTESVGLTNMKATPLDAILTPRLSPTLY

SEQ ID NO: 4 - protein, 591 aa, Artificial Sequence
  VARIANT (1)..(591): 的F6H mutant SumotrF6H
MADSEVNQEAKPEVKPEVKPETHINLKVSDGSSEIFFKIKKTTPLRRLMEAFAKRQGKEMDSLRFLYDGIRIQADQTPEDLDMEDNDIIEAHREQIGGMPKKSSLNAPPEAGGARFITGHLHLMDGRSASDKLPHINLGLLADQHGPIFTIRLGVHRAVVVSSWELAKEIFTTHDTAVMARPRLIADDYLSYDGASLGFSPYGPYWREIRKLVTTELLSARRIELQRATRVREITQFTGELYKLWEEKKDGSGRVLVDMKQWLGNLSLNLVSRMVVGKRFYGGDDSETTKRWRGVMREFFQLIGQFIPGDGLPFLRWLDLGGFEKRTRDTAYELDKIIAMWLAEYRKREYSGDDKEQCFMALMLSLVQANPTLQLHYDADTIIKATCQVLISAASDTTTVILIWVISLLLNNADVLKKVQEELDEQVGRERRVEESDISNLPYLQAVVKETMRLYPPAPFAGVRAFSEDCTVGGYHIQKGTFLIVNLWKLHRDPRVWSDDALEFKPQRFFDKKVEVKGQDFELMPFGGGRRMCPGSNLGMHMVHFVLANILQAFDITTGSTVDMTESVGLTNMKATPLDAILTPRLSPTLY

SEQ ID NO: 5 - protein, 861 aa, Artificial Sequence
  VARIANT (1)..(861): F6H mutant MBPtrF6H
MAKIEEGKLVIWINGDKGYNGLAEVGKKFEKDTGIKVTVEHPDKLEEKFPQVAATGDGPDIIFWAHDRFGGYAQSGLLAEITPDKAFQDKLYPFTWDAVRYNGKLIAYPIAVEALSLIYNKDLLPNPPKTWEEIPALDKELKAKGKSALMFNLQEPYFTWPLIAADGGYAFKYENGKYDIKDVGVDNAGAKAGLTFLVDLIKNKHMNADTDYSIAEAAFNKGETAMTINGPWAWSNIDTSKVNYGVTVLPTFKGQPSKPFVGVLSAGINAASPNKELAKEFLENYLLTDEGLEAVNKDKPLGAVALKSYEEELVKDPRIAATMENAQKGEIMPNIPQMSAFWYAVRTAVINAASGRQTVDEALKDAQTMPKKSSLNAPPEAGGARFITGHLHLMDGRSASDKLPHINLGLLADQHGPIFTIRLGVHRAVVVSSWELAKEIFTTHDTAVMARPRLIADDYLSYDGASLGFSPYGPYWREIRKLVTTELLSARRIELQRATRVREITQFTGELYKLWEEKKDGSGRVLVDMKQWLGNLSLNLVSRMVVGKRFYGGDDSETTKRWRGVMREFFQLIGQFIPGDGLPFLRWLDLGGFEKRTRDTAYELDKIIAMWLAEYRKREYSGDDKEQCFMALMLSLVQANPTLQLHYDADTIIKATCQVLISAASDTTTVILIWVISLLLNNADVLKKVQEELDEQVGRERRVEESDISNLPYLQAVVKETMRLYPPAPFAGVRAFSEDCTVGGYHIQKGTFLIVNLWKLHRDPRVWSDDALEFKPQRFFDKKVEVKGQDFELMPFGGGRRMCPGSNLGMHMVHFVLANILQAFDITTGSTVDMTESVGLTNMKATPLDAILTPRLSPTLY

SEQ ID NO: 6 - protein, 509 aa, Artificial Sequence
  VARIANT (1)..(509): F6H mutant 2B1trF6H
MAKKTSSKGKLPPGPSMPKKSSLNAPPEAGGARFITGHLHLMDGRSASDKLPHINLGLLADQHGPIFTIRLGVHRAVVVSSWELAKEIFTTHDTAVMARPRLIADDYLSYDGASLGFSPYGPYWREIRKLVTTELLSARRIELQRATRVREITQFTGELYKLWEEKKDGSGRVLVDMKQWLGNLSLNLVSRMVVGKRFYGGDDSETTKRWRGVMREFFQLIGQFIPGDGLPFLRWLDLGGFEKRTRDTAYELDKIIAMWLAEYRKREYSGDDKEQCFMALMLSLVQANPTLQLHYDADTIIKATCQVLISAASDTTTVILIWVISLLLNNADVLKKVQEELDEQVGRERRVEESDISNLPYLQAVVKETMRLYPPAPFAGVRAFSEDCTVGGYHIQKGTFLIVNLWKLHRDPRVWSDDALEFKPQRFFDKKVEVKGQDFELMPFGGGRRMCPGSNLGMHMVHFVLANILQAFDITTGSTVDMTESVGLTNMKATPLDAILTPRLSPTLY

SEQ ID NO: 7 - protein, 712 aa, Arabidopsis thaliana
MSSSSSSSTSMIDLMAAIIKGEPVIVSDPANASAYESVAAELSSMLIENRQFAMIVTTSIAVLIGCIVMLVWRRSGSGNSKRVEPLKPLVIKPREEEIDDGRKKVTIFFGTQTGTAEGFAKALGEEAKARYEKTRFKIVDLDDYAADDDEYEEKLKKEDVAFFFLATYGDGEPTDNAARFYKWFTEGNDRGEWLKNLKYGVFGLGNRQYEHFNKVAKVVDDILVEQGAQRLVQVGLGDDDQCIEDDFTAWREALWPELDTILREEGDTAVATPYTAAVLEYRVSIHDSEDAKFNDINMANGNGYTVFDAQHPYKANVAVKRELHTPESDRSCIHLEFDIAGSGLTYETGDHVGVLCDNLSETVDEALRLLDMSPDTYFSLHAEKEDGTPISSSLPPPFPPCNLRTALTRYACLLSSPKKSALVALAAHASDPTEAERLKHLASPAGKVDEYSKWVVESQRSLLEVMAEFPSAKPPLGVFFAGVAPRLQPRFYSISSSPKIAETRIHVTCALVYEKMPTGRIHKGVCSTWMKNAVPYEKSENCSSAPIFVRQSNFKLPSDSKVPIIMIGPGTGLAPFRGFLQERLALVESGVELGPSVLFFGCRNRRMDFIYEEELQRFVESGALAELSVAFSREGPTKEYVQHKMMDKASDIWNMISQGAYLYVCGDAKGMARDVHRSLHTIAQEQGSMDSTKAEGFVKNLQTSGRYLRDVW

SEQ ID NO: 8 - protein, 641 aa, Artificial Sequence
  VARIANT (1)..(641): AtCPR mutant trAtCPR
MRRSGSGNSKRVEPLKPLVIKPREEEIDDGRKKVTIFFGTQTGTAEGFAKALGEEAKARYEKTRFKIVDLDDYAADDDEYEEKLKKEDVAFFFLATYGDGEPTDNAARFYKWFTEGNDRGEWLKNLKYGVFGLGNRQYEHFNKVAKVVDDILVEQGAQRLVQVGLGDDDQCIEDDFTAWREALWPELDTILREEGDTAVATPYTAAVLEYRVSIHDSEDAKFNDINMANGNGYTVFDAQHPYKANVAVKRELHTPESDRSCIHLEFDIAGSGLTYETGDHVGVLCDNLSETVDEALRLLDMSPDTYFSLHAEKEDGTPISSSLPPPFPPCNLRTALTRYACLLSSPKKSALVALAAHASDPTEAERLKHLASPAGKVDEYSKWVVESQRSLLEVMAEFPSAKPPLGVFFAGVAPRLQPRFYSISSSPKIAETRIHVTCALVYEKMPTGRIHKGVCSTWMKNAVPYEKSENCSSAPIFVRQSNFKLPSDSKVPIIMIGPGTGLAPFRGFLQERLALVESGVELGPSVLFFGCRNRRMDFIYEEELQRFVESGALAELSVAFSREGPTKEYVQHKMMDKASDIWNMISQGAYLYVCGDAKGMARDVHRSLHTIAQEQGSMDSTKAEGFVKNLQTSGRYLRDVW

SEQ ID NO: 9 - DNA, 25 bp, Primer
tataccatggaactgagcagtgtga

SEQ ID NO: 10 - DNA, 36 bp, Primer
ctcgaattcggatccactagtttaatataaagtcgg

SEQ ID NO: 11 - DNA, 43 bp, Primer
ctttaagaaggagatataccatggcgatgccgaagaaaagctc

SEQ ID NO: 12 - DNA, 63 bp, Primer
ctttaagaaggagatataccatggctctgttattagcagtttttatgccgaagaaaagctctt

SEQ ID NO: 13 - DNA, 39 bp, Primer
ctttaagaaggagatataccatggctaaaatcgaagaag

SEQ ID NO: 14 - DNA, 35 bp, Primer
ctgaaagacgcgcagactatgccgaagaaaagctc

SEQ ID NO: 15 - DNA, 35 bp, Primer
gagcttttcttcggcatagtctgcgcgtctttcag

SEQ ID NO: 16 - DNA, 87 bp, Primer
ctttaagaaggagatataccatggctaagaaaacgagctctaaagggaagctcccaccaggacctagcatgccgaagaaaagctctt

SEQ ID NO: 17 - DNA, 44 bp, Primer
ctttaagaaggagatataccatggcggactcagaagtcaatctt

SEQ ID NO: 18 - DNA, 36 bp, Primer
gagaacagattggtggtatgccgaagaaaagctctt

SEQ ID NO: 19 - DNA, 36 bp, Primer
aagagcttttcttcggcataccaccaatctgttctc

SEQ ID NO: 20 - DNA, 27 bp, Primer
tataccatgggtgactgcgttgccccg

SEQ ID NO: 21 - DNA, 30 bp, Primer
cgggatccttacttcggcaggtcgccgctc

SEQ ID NO: 22 - DNA, 29 bp, Primer
cgggatcccttatgcgactcctgcattag

SEQ ID NO: 23 - DNA, 26 bp, Primer
gcccaagcttttatgccagcatcttc

SEQ ID NO: 24 - DNA, 31 bp, Primer
agatatacatatggttacggtggaagaatac

SEQ ID NO: 25 - DNA, 30 bp, Primer
ccgctcgagttaggtagccacactatgcag

SEQ ID NO: 26 - DNA, 30 bp, Primer
ccgctcgagctagaaataattttgtttaac

SEQ ID NO: 27 - DNA, 28 bp, Primer
gagcctaggttagttaccgattttaaag

SEQ ID NO: 28 - DNA, 38 bp, Primer
gaagatgctggcataaaagcttcgatcccgcgaaatta

SEQ ID NO: 29 - DNA, 38 bp, Primer
cgacttaagcattatgcggccgcctacgccaggttttc